European Patent Specification EP 3 269 731 B1, published October 4, 2023. Title: MOLECULAR DESIGN OF RECOMBINANT PROTEIN DRUG. Applicant: Tsinghua University Beijing Protgen Ltd. The sequence listing filed with the application follows.

SEQUENCE LISTING (39 sequences)

SEQ ID NO: 1 - protein, 183 aa, Homo sapiens
HSHRDFQPVLHLVALNSPLSGGMRGIRGADFQCFQQARAVGLAGTFRAFLSSRLQDLYSIVRRADRAAVPIVNLKDELLFPSWEALFSGSEGPLKPGARIFSFDGKDVLRHPTWPQKSVWHGSDPNGRRLTESYCETWRTEAPSATGQASSLLGGRLLGQSAASCHHAYIVLCIENSFMTASK

SEQ ID NO: 2 - protein, 192 aa, artificial sequence
  mutant
MGGSHHHHHHSHRDFQPVLHLVALNSPLSGGMRGIRGADFQCFQQARAVGLAGTFRAFLSSRLQDLYSIVRRADRAAVPIVNLKDELLFPSWEALFSGSEGPLKPGARIFSFDGKDVLRHPTWPQKSVWHGSDPNGRRLTESYCETWRTEAPSATGQASSLLGGRLLGQSAASCHHAYIVLCIENSFMTASK

SEQ ID NO: 3 - protein, 180 aa, artificial sequence
  mutant
DFQPVLHLVALNSPLSGGMRGIRGADFQCFQQARAVGLAGTFRAFLSSRLQDLYSIVRRADRAAVPIVNLKDELLFPSWEALFSGESGAGKTPGARIFSFDGKDVLRHPTWPQKSVWHGSDPNGRRLTESYCETWRTEAPSATGQASSLLGGRLLGQSAASCHHAYIVLCIENSFMTASK

SEQ ID NO: 4 - protein, 171 aa, artificial sequence
  mutant
DFQPVLHLVALNSPLSGGMRGIRGADFQCFQQARAVGLAGTFRAFLSSRLQDLYSIVRRADRAAVPIVNLKDELLFPSWEALFSGSEGPLKSPGARIFSFDGKDVLRHPTWPQKSVWHGSDPNGRRLTESYCETWRTEAPSATGQASSLLGGRLLGQSAASCHHAYIVLCI

SEQ ID NO: 5 - protein, 171 aa, artificial sequence
  mutant
DFQPVLHLVALNSPLSGGMRGIRGADFQCFQQARAVGLAGTFRAFLSSRLQDLYSIVRRADRAAVPIVNLKDELLFPSWEALFSGSEGPLKTPGARIFSFDGKDVLRHPTWPQKSVWHGSDPNGRRLTESYCETWRTEAPSATGQASSLLGGRLLGQSAASCHHAYIVLCI

SEQ ID NO: 6 - protein, 171 aa, artificial sequence
  mutant
DFQPVLHLVALNSPLSGGMRGIRGADFQCFQQARAVGLAGTFRAFLSSRLQDLYSIVRRADRAAVPIVNLKDELLFPSWEALFSGESGAGKTPGARIFSFDGKDVLRHPTWPQKSVWHGSDPNGRRLTESYCETWRTEAPSATGQASSLLGGRLLGQSAASCHHAYIVLCI

SEQ ID NO: 7 - protein, 177 aa, artificial sequence
  mutant
HSHRDFQPVLHLVALNSPLSGGMRGIRGADFQCFQQARAVGLAGTFRAFLSSRLQDLYSIVRRADRAAVPIVNLKDELLFPSWEALFSGESGAGKTPGARIFSFDGKDVLRHPTWPQKSVWHGSDPNGRRLTESYCETWRTEAPSATGQASSLLGGRLLGQSAASCHHAYIVLCIEN

SEQ ID NO: 8 - protein, 180 aa, artificial sequence
  mutant
HSHRDFQPVLHLVALNSPLSGGMRGIRGADFQCFQQARAVGLAGTFRAFLSSRLQDLYSIVRRADRAAVPIVNLKDELLFPSWEALFSGESGAGKTPGARIFSFDGKDVLRHPTWPQKSVWHGSDPNGRRLTESYCETWRTEAPSATGQASSLLGGRLLGQSAASCHHAYIVLCIENSFM

SEQ ID NO: 9 - protein, 176 aa, artificial sequence
  mutant
HSHRDFQPVLHLVALNSPLSGGMRGIRGADFQCFQQARAVGLAGTFRAFLSSRLQDLYSIVRRADRAAVPIVNLKDELLFPSWEALFSGSEGPLKPGARIFSFDGKDVLRHPTWPQKSVWHGSDPNGRRLTESYCETWRTEAPSATGQASSLLGGRLLGQSAASCHHAYIVLCIEN

SEQ ID NO: 10 - protein, 175 aa, artificial sequence
  mutant
HRDFQPVLHLVALNSPLSGGMRGIRGADFQCFQQARAVGLAGTFRAFLSSRLQDLYSIVRRADRAAVPIVNLKDELLFPSWEALFSGESGAGKTPGARIFSFDGKDVLRHPTWPQKSVWHGSDPNGRRLTESYCETWRTEAPSATGQASSLLGGRLLGQSAASCHHAYIVLCIEN

SEQ ID NO: 11 - protein, 178 aa, artificial sequence
  mutant
HRDFQPVLHLVALNSPLSGGMRGIRGADFQCFQQARAVGLAGTFRAFLSSRLQDLYSIVRRADRAAVPIVNLKDELLFPSWEALFSGESGAGKTPGARIFSFDGKDVLRHPTWPQKSVWHGSDPNGRRLTESYCETWRTEAPSATGQASSLLGGRLLGQSAASCHHAYIVLCIENSFM

SEQ ID NO: 12 - protein, 181 aa, artificial sequence
  mutant
HRDFQPVLHLVALNSPLSGGMRGIRGADFQCFQQARAVGLAGTFRAFLSSRLQDLYSIVRRADRAAVPIVNLKDELLFPSWEALFSGESGAGKTPGARIFSFDGKDVLRHPTWPQKSVWHGSDPNGRRLTESYCETWRTEAPSATGQASSLLGGRLLGQSAASCHHAYIVLCIENSFMTAS

SEQ ID NO: 13 - protein, 182 aa, artificial sequence
  mutant
SHRDFQPVLHLVALNSPLSGGMRGIRGADFQCFQQARAVGLAGTFRAFLSSRLQDLYSIVRRADRAAVPIVNLKDELLFPSWEALFSGESGAGKTPGARIFSFDGKDVLRHPTWPQKSVWHGSDPNGRRLTESYCETWRTEAPSATGQASSLLGGRLLGQSAASCHHAYIVLCIENSFMTAS

SEQ ID NO: 14 - protein, 176 aa, artificial sequence
  mutant
SHRDFQPVLHLVALNSPLSGGMRGIRGADFQCFQQARAVGLAGTFRAFLSSRLQDLYSIVRRADRAAVPIVNLKDELLFPSWEALFSGESGAGKTPGARIFSFDGKDVLRHPTWPQKSVWHGSDPNGRRLTESYCETWRTEAPSATGQASSLLGGRLLGQSAASCHHAYIVLCIEN

SEQ ID NO: 15 - protein, 179 aa, artificial sequence
  mutant
SHRDFQPVLHLVALNSPLSGGMRGIRGADFQCFQQARAVGLAGTFRAFLSSRLQDLYSIVRRADRAAVPIVNLKDELLFPSWEALFSGESGAGKTPGARIFSFDGKDVLRHPTWPQKSVWHGSDPNGRRLTESYCETWRTEAPSATGQASSLLGGRLLGQSAASCHHAYIVLCIENSFM

SEQ ID NO: 16 - protein, 183 aa, artificial sequence
  mutant
SHRDFQPVLHLVALNSPLSGGMRGIRGADFQCFQQARAVGLAGTFRAFLSSRLQDLYSIVRRADRAAVPIVNLKDELLFPSWEALFSGESGAGKTPGARIFSFDGKDVLRHPTWPQKSVWHGSDPNGRRLTESYCETWRTEAPSATGQASSLLGGRLLGQSAASCHHAYIVLCIENSFMTASK

SEQ ID NO: 17 - protein, 182 aa, artificial sequence
  mutant
HRDFQPVLHLVALNSPLSGGMRGIRGADFQCFQQARAVGLAGTFRAFLSSRLQDLYSIVRRADRAAVPIVNLKDELLFPSWEALFSGESGAGKTPGARIFSFDGKDVLRHPTWPQKSVWHGSDPNGRRLTESYCETWRTEAPSATGQASSLLGGRLLGQSAASCHHAYIVLCIENSFMTASK

SEQ ID NO: 18 - protein, 183 aa, artificial sequence
  mutant
HSHRDFQPVLHLVALNSPLSGGMRGIRGADFQCFQQARAVGLAGTFRAFLSSRLQDLYSIVRRADRAAVPIVNLKDELLFPSWEALFGESGAGKTPGARIFSFDGKDVLRHPTWPQKSVWHGSDPNGRRLTESYCETWRTEAPSATGQASSLLGGRLLGQSAASCHHAYIVLCIENSFMTASK

SEQ ID NO: 19 - protein, 183 aa, artificial sequence
  mutant
HSHRDFQPVLHLVALNSPLSGGMRGIRGADFQCFQQARAVGLAGTFRAFLSSRLQDLYSIVRRADRAAVPIVNLKDELLFPSWEALFSGESGAGKTPARIFSFDGKDVLRHPTWPQKSVWHGSDPNGRRLTESYCETWRTEAPSATGQASSLLGGRLLGQSAASCHHAYIVLCIENSFMTASK

SEQ ID NO: 20 - protein, 183 aa, artificial sequence
  mutant
HSHRDFQPVLHLVALNSPLSGGMRGIRGADFQCFQQARAVGLAGTFRAFLSSRLQDLYSIVRRADRAAVPIVNLKDELLFPSWEALFSGESGAGKTGARIFSFDGKDVLRHPTWPQKSVWHGSDPNGRRLTESYCETWRTEAPSATGQASSLLGGRLLGQSAASCHHAYIVLCIENSFMTASK

SEQ ID NO: 21 - protein, 184 aa, artificial sequence
  mutant
HSHRDFQPVLHLVALNSPLSGGMRGIRGADFQCFQQARAVGLAGTFRAFLSSRLQDLYSIVRRADRAAVPIVNLKDELLFPSWEALFSGESGAGKTGGARIFSFDGKDVLRHPTWPQKSVWHGSDPNGRRLTESYCETWRTEAPSATGQASSLLGGRLLGQSAASCHHAYIVLCIENSFMTASK

SEQ ID NO: 22 - protein, 183 aa, artificial sequence
  mutant
HSHRDFQPVLHLVALNSPLSGGMRGIRGADFQCFQQARAVGLAGTFRAFLSSRLQDLYSIVRRADRAAVPIVNLKDELLFPSWEALFSGSEGPLKPGARIFSFDGKDVLRHPTWPQKSVWHGSDPNGRRLTESYCETWRTEAPSATGQASSLLGGRLLGQSAASCHHAYIVLCIANSFMTASK

SEQ ID NO: 23 - protein, 183 aa, artificial sequence
  mutant
HSHRDFQPVLHLVALNSPLSGGMRGIRGADFQCFQQARAVGLAGTFRAFLSSRLQDLYSIVRRADRAAVPIVNLKDELLFPSWEALFSGSEGPLKPGARIFSFDGKDVLRHPTWPQKSVWHGSDPNGRRLTESYCETWRTEAPSATGQASSLLGGRLLGQSAASCHHAYIVLEIENSFMTASK

SEQ ID NO: 24 - protein, 184 aa, artificial sequence
  mutant
HSHRDFQPVLHLVALNSPLSGGMRGIRGADFQCFQQARAVGLAGTFRAFLSSRLQDLYSIVRRADRAAVPIVNLKDELLFPSWEALFSGESGAGKTPGARIFSFDGKDVLRHPTWPQKSVWHGSDPNGRRLTESYCETWRTEAPSATGQASSLLGGRLLGQSAASCHHAYIVLCIENSFMTASK

SEQ ID NO: 25 - protein, 179 aa, artificial sequence
  mutant
RDFQPVLHLVALNSPLSGGMRGIRGADFQCFQQARQVGLAGTFRAFLSSRLQDLYSIVRRADRAAVPIVNLKDELLFPSWEALFSSEGPLKPGARIFSFDGKDVLRHPTWPQKSVWHGSDPNGRRLTESYCETWRTEAPSATGQASSLLGGRLLGQSAASCHHAYIVLCIENSFMTASK

SEQ ID NO: 26 - protein, 180 aa, artificial sequence
  mutant
RDFQPVLHLVALNSPLSGGMRGIRGADFQCFQQARAVGLAGTFRAFLSSRLQDLYSIVRRADRGSVPIVNLKDEVLSPSWDSLFSGSQGQLQPGARIFSFDGRDILQDSAWPQKSVWHGSDAKGRRLPESYCEAWRTDERGTSGQASSLLSGRLLEQKAASCHNSYIVLCIENSFMTASK

SEQ ID NO: 27 - protein, 184 aa, artificial sequence
  mutant
HVHQDFQPALHLVALNTPLSGGMRGIRGADFQCFQQARQVGLAGTFRAFLSSRLQDLYSIVRRADRTAVPIVNLRDEVLFSNWEALFTGSEAPLRAGARIFSFDGRDVLRHPTWPQKSVWHGSDPNGRRLTESYCETWRTEAPSATGQASSLLAGRLLEQKAAGCHNAFIVLCIENSFMTSSSK

SEQ ID NO: 28 - protein, 185 aa, artificial sequence
  mutant
HTHQDFHPVLHLVALNTPLSGGMRGIRGADFQCFQQARAVGLSGTFRAFLSSRLQDLYSIVRRADRAAVPIVNLKDELLFPSWEALFSGESGAGKTGGARIFSFDGRDVLRHPAWPQKSVWHGSDPSGRRLTESYCETWRTDSRAATGQASSLLAGRLLEQKAAGCHNAFIVLCIENSFMTSSSK

SEQ ID NO: 29 - protein, 183 aa, artificial sequence
  mutant
HSHRDFQPVLHLVALNSPLSGGMRGIRGADFQCFQQARAVGLAGTFRAFLSSRLQDLYSIVRRADRAAVPIVNLKDELLFPSWEALFSGSEGPLKPGARIFSFDGRDVLRHPTWPQKSVWHGSDPSGHRLTESYCETWRTDSRAATGQASSLLGGRLLGQSAASCHHAYIVLCIANSFMTASK

SEQ ID NO: 30 - protein, 179 aa, artificial sequence
  mutant
DFQPVLHLVALNSPLSGGMRGIRGADFQCFQQARAVGLAGTFRAFLSSRLQDLYSIVRRADRAAVPIVNLKDELLFPSWEALFSGSEGPLRPGARIFSFDGKDVLRHPTLPQKSVWHGSDPSGRRLTESYCETWRTDSRAATGQASSLLGGRLLGQSAASCHHAYIVLCIENSFMTASK

SEQ ID NO: 31 - protein, 180 aa, artificial sequence
  mutant
DFQPVLHLVALNSPLSGGMRGIRGADFQCFQQARAVGLAGTFRAFLSSRLQDLYSIVRRADRAAVPIVNLKDELLFPSWEALFSGSEGPLRPGARIFSFDGKDVLRHPTLPQKSVWHGSDPSGRRLTESYCETWRTDSRAATGQASSLLGGRLLGQSAASCHHAYIVLCIENSFMTASKK

SEQ ID NO: 32 - protein, 184 aa, artificial sequence
  mutant
HTHQDFHPVLHLVALNTPLSGGMRGIRGADFQCFQQARAVGLAGTFRAFLSSRLQDLYSIVRRADRAAVPIVNLKDELLFPSWEALFSGSEGPLKPGARIFSFDGRDILQDSAWPQKSVWHGSDPNGRRLTESYCETWRTEAPSATGQASSLSSGKLLEQSVSSCQHAFVVLCIENSFMTAAKK

SEQ ID NO: 33 - protein, 183 aa, artificial sequence
  mutant
TPTWYPRMLRVAALNEPSTGDLQGIRGADFQCFQQARAVGLSGTFRAFLSSRLQDLYSIVRRADRAAVPIVNLKDEVLSPSWDSLFSGSQGQLQPGARIFSFDGKDVLRHPTWPQKSVWHGSDPSGRRLMESYCETWRTETTGATGQASSLLGGRLLGQSAASCHHAYIVLCIENSFMTNNRK

SEQ ID NO: 34 - protein, 182 aa, artificial sequence
  mutant
HTHTSGPGLHLIALNSPQVGNMRGIRGADFQCFQQARAVGLAGTFRAFLSSRLQDLYSIVRRADRSSVPIVNLKDEVLSPSWDSLFSVSQGQLQPGARIFSFDGRDILQDSAWPQKSVWHGSDPNGRRLTESYCETWRTEAPSATGQASSLLGGRLLGQSAASCHHAYIVLCIENSFMTASK

SEQ ID NO: 35 - DNA, 31 bp, artificial sequence
  primer
ggaattccatatgcacagccaccgcgacttc

SEQ ID NO: 36 - DNA, 34 bp, artificial sequence
  primer
ccgctcgagttacttggaggcagtcatgaagctg

SEQ ID NO: 37 - protein, 193 aa, artificial sequence
  mutant
MGGSHHHHHHSHRDFQPVLHLVALNSPLSGGMRGIRGADFQCFQQARAVGLAGTFRAFLSSRLQDLYSIVRRADRAAVPIVNLKDELLFPSWEALFSGESGAGKTPGARIFSFDGKDVLRHPTWPQKSVWHGSDPNGRRLTESYCETWRTEAPSATGQASSLLGGRLLGQSAASCHHAYIVLCIENSFMTASK

SEQ ID NO: 38 - protein, 192 aa, artificial sequence
  mutant
MGGSHHHHHHSHRDFQPVLHLVALNSPLSGGMRGIRGADFQCFQQARAVGLAGTFRAFLSSRLQDLYSIVRRADRAAVPIVNLKDELLFPSWEALFSGSEGPLKPGARIFSFDGRDVLRHPTWPQKSVWHGSDPSGHRLTESYCETWRTDSRAATGQASSLLGGRLLGQSAASCHHAYIVLCIANSFMTASK

SEQ ID NO: 39 - protein, 194 aa, artificial sequence
  mutant
MGGSHHHHHHTHQDFHPVLHLVALNTPLSGGMRGIRGADFQCFQQARAVGLSGTFRAFLSSRLQDLYSIVRRADRAAVPIVNLKDELLFPSWEALFSGESGAGKTGGARIFSFDGRDVLRHPAWPQKSVWHGSDPSGRRLTESYCETWRTDSRAATGQASSLLAGRLLEQKAAGCHNAFIVLCIENSFMTSSSK